European Patent Application EP 4 257 666 A1, published October 11, 2023. Title: An amplification method of nucleic acid and thermal cycler. Applicant: YAMAGUCHI UNIVERSITY YANAGIYA MACHINERY CO., LTD. The sequence listing filed with the application follows.

SEQUENCE LISTING (8 sequences)

SEQ ID NO: 1 - DNA, 711 bp, artificial
  EGFP
  misc_feature: Inventor:  Fujimoto Tetsunori; Nakata Noriatsu; Nakatomi Tadashi; Akada Rinji
atggtgagcaaaggtgaagaactgtttaccggtgttgttccgattctggttgaactggatggtgatgttaatggccacaaattttcagttagcggtgaaggcgaaggtgatgcaacctatggtaaactgaccctgaaatttatctgtaccaccggcaaactgccggttccgtggccgaccctggttaccaccctgacctatggtgttcagtgttttagccgttatccggatcatatgaaacagcacgattttttcaaaagcgcaatgccggaaggttatgttcaagaacgtaccatcttcttcaaagatgacggcaactataaaacccgtgccgaagttaaatttgaaggtgataccctggtgaatcgcattgaactgaaaggcatcgattttaaagaggatggtaatatcctgggccacaaactggaatataattataatagccacaacgtgtacatcatggccgacaaacagaaaaatggcatcaaagtgaacttcaaaatccgccacaatattgaagatggttcagttcagctggcagatcattatcagcagaataccccgattggtgatggtccggttctgctgccggataatcattatctgagcacccagagcgcactgagcaaagatccgaatgaaaaacgtgatcacatggtgctgctggaatttgttaccgcagcaggtattaccctgggtatggatgaataa

SEQ ID NO: 2 - DNA, 2328 bp, Pyrococcus furiosus
atgatcctggacgttgactacatcaccgaagaaggtaaaccggttatccgtctgttcaaaaaagaaaacggtaaattcaaaatcgaacacgaccgtaccttccgtccgtacatctacgctctgctgcgtgacgactccaaaatcgaagaagttaaaaaaatcaccggtgaacgtcacggtaaaatcgttcgtatcgttgacgttgaaaaagttgaaaaaaaattcctgggtaaaccgatcaccgtttggaaactgtacctggaacacccgcaggacgttccgaccatccgtgaaaaagttcgtgaacacccggctgttgttgacatcttcgaatacgacatcccgttcgctaaacgttacctgatcgacaaaggtctgatcccgatggaaggtgaagaagaactgaaaatcctggctttcgacatcgaaaccctgtaccacgaaggtgaagaattcggtaaaggtccgatcatcatgatctcctacgctgacgaaaacgaagctaaagttatcacctggaaaaacatcgacctgccgtacgttgaagttgtttcctccgaacgtgaaatgatcaaacgtttcctgcgtatcatccgtgaaaaagacccggacatcatcgttacctacaacggtgactccttcgacttcccgtacctggctaaacgtgctgaaaaactgggtatcaaactgaccatcggtcgtgacggttccgaaccgaaaatgcagcgtatcggtgacatgaccgctgttgaagttaaaggtcgtatccacttcgacctgtaccacgttatcacccgtaccatcaacctgccgacctacaccctggaagctgtttacgaagctatcttcggtaaaccgaaagaaaaagtttacgctgacgaaatcgctaaagcttgggaatccggtgaaaacctggaacgtgttgctaaatactccatggaagacgctaaagctacctacgaactgggtaaagaattcctgccgatggaaatccagctgtcccgtctggttggtcagccgctgtgggacgtttcccgttcctccaccggtaacctggttgaatggttcctgctgcgtaaagcttacgaacgtaacgaagttgctccgaacaaaccgtccgaagaagaataccagcgtcgtctgcgtgaatcctacaccggtggtttcgttaaagaaccggaaaaaggtctgtgggaaaacatcgtttacctggacttccgtgctctgtacccgtccatcatcatcacccacaacgtttccccggacaccctgaacctggaaggttgcaaaaactacgacatcgctccgcaggttggtcacaaattctgcaaagacatcccgggtttcatcccgtccctgctgggtcacctgctggaagaacgtcagaaaatcaaaaccaaaatgaaagaaacccaggacccgatcgaaaaaatcctgctggactaccgtcagaaagctatcaaactgctggctaactccttctacggttactacggttacgctaaagctcgttggtactgcaaagaatgcgctgaatccgttaccgcttggggtcgtaaatacatcgaactggtttggaaagaactggaagaaaaattcggtttcaaagttctgtacatcgacaccgacggtctgtacgctaccatcccgggtggtgaatccgaagaaatcaaaaaaaaagctctggaattcgttaaatacatcaactccaaactgccgggtctgctggaactggaatacgaaggtttctacaaacgtggtttcttcgttaccaaaaaacgttacgctgttatcgacgaagaaggtaaagttatcacccgtggtctggaaatcgttcgtcgtgactggtccgaaatcgctaaagaaacccaggctcgtgttctggaaaccatcctgaaacacggtgacgttgaagaagctgttcgtatcgttaaagaagttatccagaaactggctaactacgaaatcccgccggaaaaactggctatctacgaacagatcacccgtccgctgcacgaatacaaagctatcggtccgcacgttgctgttgctaaaaaactggctgctaaaggtgttaaaatcaaaccgggtatggttatcggttacatcgttctgcgtggtgacggtccgatctccaaccgtgctatcctggctgaagaatacgacccgaaaaaacacaaatacgacgctgaatactacatcgaaaaccaggttctgccggctgttctgcgtatcctggaaggtttcggttaccgtaaagaagacctgcgttaccagaaaacccgtcaggttggtctgacctcctggctgaacatcaaaaaatcctaa

SEQ ID NO: 3 - DNA, 30 bp, artificial
  forward primer
atggtgagcaaaggtgaagaactgtttacc

SEQ ID NO: 4 - DNA, 30 bp, artificial
  riverse primer
gcaggtattaccctgggtatggatgaataa

SEQ ID NO: 5 - DNA, 7609 bp, Homo sapiens
gacggatcgggagatctcccgatcccctatggtcgactctcagtacaatctgctctgatgccgcatagttaagccagtatctgctccctgcttgtgtgttggaggtcgctgagtagtgcgcgagcaaaatttaagctacaacaaggcaaggcttgaccgacaattgcatgaagaatctgcttagggttaggcgttttgcgctgcttcgcgatgtacgggccagatatacgcgttgacattgattattgactagttattaatagtaatcaattacggggtcattagttcatagcccatatatggagttccgcgttacataacttacggtaaatggcccgcctggctgaccgcccaacgacccccgcccattgacgtcaataatgacgtatgttcccatagtaacgccaatagggactttccattgacgtcaatgggtggactatttacggtaaactgcccacttggcagtacatcaagtgtatcatatgccaagtacgccccctattgacgtcaatgacggtaaatggcccgcctggcattatgcccagtacatgaccttatgggactttcctacttggcagtacatctacgtattagtcatcgctattaccatggtgatgcggttttggcagtacatcaatgggcgtggatagcggtttgactcacggggatttccaagtctccaccccattgacgtcaatgggagtttgttttggcaccaaaatcaacgggactttccaaaatgtcgtaacaactccgccccattgacgcaaatgggcggtaggcgtgtacggtgggaggtctatataagcagagctctctggctaactagagaacccactgcttactggcttatcgaaattaatacgactcactatagggagacccaagcttggtaccgagctcggatccgatgtgggtgaccaaactcctgccagccctgctgctgcagcatgtcctcctgcatctcctcctgctccccatcgccatcccctatgcagagggacaaaggaaaagaagaaatacaattcatgaattcaaaaaatcagcaaagactaccctaatcaaaatagatccagcactgaagataaaaaccaaaaaagtgaatactgcagaccaatgtgctaatagatgtactaggaataaaggacttccattcacttgcaaggcttttgtttttgataaagcaagaaaacaatgcctctggttccccttcaatagcatgtcaagtggagtgaaaaaagaatttggccatgaatttgacctctatgaaaacaaagactacattagaaactgcatcattggtaaaggacgcagctacaagggaacagtatctatcactaagagtggcatcaaatgtcagccctggagttccatgataccacacgaacacagctttttgccttcgagctatcggggtaaagacctacaggaaaactactgtcgaaatcctcgaggggaagaagggggaccctggtgtttcacaagcaatccagaggtacgctacgaagtctgtgacattcctcagtgttcagaagttgaatgcatgacctgcaatggggagagttatcgaggtctcatggatcatacagaatcaggcaagatttgtcagcgctgggatcatcagacaccacaccggcacaaattcttgcctgaaagatatcccgacaagggctttgatgataattattgccgcaatcccgatggccagccgaggccatggtgctatactcttgaccctcacacccgctgggagtactgtgcaattaaaacatgcgctgacaatactatgaatgacactgatgttcctttggaaacaactgaatgcatccaaggtcaaggagaaggctacaggggcactgtcaataccatttggaatggaattccatgtcagcgttgggattctcagtatcctcacgagcatgacatgactcctgaaaatttcaagtgcaaggacctacgagaaaattactgccgaaatccagatgggtctgaatcaccctggtgttttaccactgatccaaacatccgagttggctactgctcccaaattccaaactgtgatatgtcacatggacaagattgttatcgtgggaatggcaaaaattatatgggcaacttatcccaaacaagatctggactaacatgttcaatgtgggacaagaacatggaagacttacatcgtcatatcttctgggaaccagatgcaagtaagctgaatgagaattactgccgaaatccagatgatgatgctcatggaccctggtgctacacgggaaatccactcattccttgggattattgccctatttctcgttgtgaaggtgataccacacctacaatagtcaatttagaccatcccgtaatatcttgtgccaaaacgaaacaattgcgagttgtaaatgggattccaacacgaacaaacataggatggatggttagtttgagatacagaaataaacatatctgcggaggatcattgataaaggagagttgggttcttactgcacgacagtgtttcccttctcgagacttgaaagattatgaagcttggcttggaattcatgatgtccacggaagaggagatgagaaatgcaaacaggttctcaatgtttcccagctggtatatggccctgaaggatcagatctggttttaatgaagcttgccaggcctgctgtcctggatgattttgttagtacgattgatttacctaattatggatgcacaattcctgaaaagaccagttgcagtgtttatggctggggctacactggattgatcaactatgatggcctattacgagtggcacatctctatataatgggaaatgagaaatgcagccagcatcatcgagggaaggtgactctgaatgagtctgaaatatgtgctggggctgaaaagattggatcaggaccatgtgagggggattatggtggcccacttgtttgtgagcaacataaaatgagaatggttcttggtgtcattgttcctggtcgtggatgtgccattccaaatcgtcctggtatttttgtccgagtagcatattatgcaaaatggatacacaaaattattttaacatataaggtaccacagtcataggaattctgcagatatccatcacactggcggccgctcgagcatgcatctagagggccctattctatagtgtcacctaaatgctagagctcgctgatcagcctcgactgtgccttctagttgccagccatctgttgtttgcccctcccccgtgccttccttgaccctggaaggtgccactcccactgtcctttcctaataaaatgaggaaattgcatcgcattgtctgagtaggtgtcattctattctggggggtggggtggggcaggacagcaagggggaggattgggaagacaatagcaggcatgctggggatgcggtgggctctatggcttctgaggcggaaagaaccagctggggctctagggggtatccccacgcgccctgtagcggcgcattaagcgcggcgggtgtggtggttacgcgcagcgtgaccgctacacttgccagcgccctagcgcccgctcctttcgctttcttcccttcctttctcgccacgttcgccggctttccccgtcaagctctaaatcggggcatccctttagggttccgatttagtgctttacggcacctcgaccccaaaaaacttgattagggtgatggttcacgtagtgggccatcgccctgatagacggtttttcgccctttgacgttggagtccacgttctttaatagtggactcttgttccaaactggaacaacactcaaccctatctcggtctattcttttgatttataagggattttggggatttcggcctattggttaaaaaatgagctgatttaacaaaaatttaacgcgaattaattctgtggaatgtgtgtcagttagggtgtggaaagtccccaggctccccaggcaggcagaagtatgcaaagcatgcatctcaattagtcagcaaccaggtgtggaaagtccccaggctccccagcaggcagaagtatgcaaagcatgcatctcaattagtcagcaaccatagtcccgcccctaactccgcccatcccgcccctaactccgcccagttccgcccattctccgccccatggctgactaattttttttatttatgcagaggccgaggccgcctctgcctctgagctattccagaagtagtgaggaggcttttttggaggcctaggcttttgcaaaaagctcccgggagcttgtatatccattttcggatctgatcaagagacaggatgaggatcgtttcgcatgattgaacaagatggattgcacgcaggttctccggccgcttgggtggagaggctattcggctatgactgggcacaacagacaatcggctgctctgatgccgccgtgttccggctgtcagcgcaggggcgcccggttctttttgtcaagaccgacctgtccggtgccctgaatgaactgcaggacgaggcagcgcggctatcgtggctggccacgacgggcgttccttgcgcagctgtgctcgacgttgtcactgaagcgggaagggactggctgctattgggcgaagtgccggggcaggatctcctgtcatctcaccttgctcctgccgagaaagtatccatcatggctgatgcaatgcggcggctgcatacgcttgatccggctacctgcccattcgaccaccaagcgaaacatcgcatcgagcgagcacgtactcggatggaagccggtcttgtcgatcaggatgatctggacgaagagcatcaggggctcgcgccagccgaactgttcgccaggctcaaggcgcgcatgcccgacggcgaggatctcgtcgtgacccatggcgatgcctgcttgccgaatatcatggtggaaaatggccgcttttctggattcatcgactgtggccggctgggtgtggcggaccgctatcaggacatagcgttggctacccgtgatattgctgaagagcttggcggcgaatgggctgaccgcttcctcgtgctttacggtatcgccgctcccgattcgcagcgcatcgccttctatcgccttcttgacgagttcttctgagcgggactctggggttcgaaatgaccgaccaagcgacgcccaacctgccatcacgagatttcgattccaccgccgccttctatgaaaggttgggcttcggaatcgttttccgggacgccggctggatgatcctccagcgcggggatctcatgctggagttcttcgcccaccccaacttgtttattgcagcttataatggttacaaataaagcaatagcatcacaaatttcacaaataaagcatttttttcactgcattctagttgtggtttgtccaaactcatcaatgtatcttatcatgtctgtataccgtcgacctctagctagagcttggcgtaatcatggtcatagctgtttcctgtgtgaaattgttatccgctcacaattccacacaacatacgagccggaagcataaagtgtaaagcctggggtgcctaatgagtgagctaactcacattaattgcgttgcgctcactgcccgctttccagtcgggaaacctgtcgtgccagctgcattaatgaatcggccaacgcgcggggagaggcggtttgcgtattgggcgctcttccgcttcctcgctcactgactcgctgcgctcggtcgttcggctgcggcgagcggtatcagctcactcaaaggcggtaatacggttatccacagaatcaggggataacgcaggaaagaacatgtgagcaaaaggccagcaaaaggccaggaaccgtaaaaaggccgcgttgctggcgtttttccataggctccgcccccctgacgagcatcacaaaaatcgacgctcaagtcagaggtggcgaaacccgacaggactataaagataccaggcgtttccccctggaagctccctcgtgcgctctcctgttccgaccctgccgcttaccggatacctgtccgcctttctcccttcgggaagcgtggcgctttctcaatgctcacgctgtaggtatctcagttcggtgtaggtcgttcgctccaagctgggctgtgtgcacgaaccccccgttcagcccgaccgctgcgccttatccggtaactatcgtcttgagtccaacccggtaagacacgacttatcgccactggcagcagccactggtaacaggattagcagagcgaggtatgtaggcggtgctacagagttcttgaagtggtggcctaactacggctacactagaaggacagtatttggtatctgcgctctgctgaagccagttaccttcggaaaaagagttggtagctcttgatccggcaaacaaaccaccgctggtagcggtggtttttttgtttgcaagcagcagattacgcgcagaaaaaaaggatctcaagaagatcctttgatcttttctacggggtctgacgctcagtggaacgaaaactcacgttaagggattttggtcatgagattatcaaaaaggatcttcacctagatccttttaaattaaaaatgaagttttaaatcaatctaaagtatatatgagtaaacttggtctgacagttaccaatgcttaatcagtgaggcacctatctcagcgatctgtctatttcgttcatccatagttgcctgactccccgtcgtgtagataactacgatacgggagggcttaccatctggccccagtgctgcaatgataccgcgagacccacgctcaccggctccagatttatcagcaataaaccagccagccggaagggccgagcgcagaagtggtcctgcaactttatccgcctccatccagtctattaattgttgccgggaagctagagtaagtagttcgccagttaatagtttgcgcaacgttgttgccattgctacaggcatcgtggtgtcacgctcgtcgtttggtatggcttcattcagctccggttcccaacgatcaaggcgagttacatgatcccccatgttgtgcaaaaaagcggttagctccttcggtcctccgatcgttgtcagaagtaagttggccgcagtgttatcactcatggttatggcagcactgcataattctcttactgtcatgccatccgtaagatgcttttctgtgactggtgagtactcaaccaagtcattctgagaatagtgtatgcggcgaccgagttgctcttgcccggcgtcaatacgggataataccgcgccacatagcagaactttaaaagtgctcatcattggaaaacgttcttcggggcgaaaactctcaaggatcttaccgctgttgagatccagttcgatgtaacccactcgtgcacccaactgatcttcagcatcttttactttcaccagcgtttctgggtgagcaaaaacaggaaggcaaaatgccgcaaaaaagggaataagggcgacacggaaatgttgaatactcatactcttcctttttcaatattattgaagcatttatcagggttattgtctcatgagcggatacatatttgaatgtatttagaaaaataaacaaataggggttccgcgcacatttccccgaaaagtgccacctgacgtc

SEQ ID NO: 6 - DNA, 35 bp, artificial
  forward primer eCMV-600(35)
gtaatcaattacggggtcattagttcatagcccat

SEQ ID NO: 7 - DNA, 35 bp, artificial
  riverse primer BGHpA+225c(35)
ccatagagcccaccgcatccccagcatgcctgcta

SEQ ID NO: 8 - DNA, 3167 bp, artificial
  PCR product
gtaatcaattacggggtcattagttcatagcccatatatggagttccgcgttacataacttacggtaaatggcccgcctggctgaccgcccaacgacccccgcccattgacgtcaataatgacgtatgttcccatagtaacgccaatagggactttccattgacgtcaatgggtggactatttacggtaaactgcccacttggcagtacatcaagtgtatcatatgccaagtacgccccctattgacgtcaatgacggtaaatggcccgcctggcattatgcccagtacatgaccttatgggactttcctacttggcagtacatctacgtattagtcatcgctattaccatggtgatgcggttttggcagtacatcaatgggcgtggatagcggtttgactcacggggatttccaagtctccaccccattgacgtcaatgggagtttgttttggcaccaaaatcaacgggactttccaaaatgtcgtaacaactccgccccattgacgcaaatgggcggtaggcgtgtacggtgggaggtctatataagcagagctctctggctaactagagaacccactgcttactggcttatcgaaattaatacgactcactatagggagacccaagcttggtaccgagctcggatccgatgtgggtgaccaaactcctgccagccctgctgctgcagcatgtcctcctgcatctcctcctgctccccatcgccatcccctatgcagagggacaaaggaaaagaagaaatacaattcatgaattcaaaaaatcagcaaagactaccctaatcaaaatagatccagcactgaagataaaaaccaaaaaagtgaatactgcagaccaatgtgctaatagatgtactaggaataaaggacttccattcacttgcaaggcttttgtttttgataaagcaagaaaacaatgcctctggttccccttcaatagcatgtcaagtggagtgaaaaaagaatttggccatgaatttgacctctatgaaaacaaagactacattagaaactgcatcattggtaaaggacgcagctacaagggaacagtatctatcactaagagtggcatcaaatgtcagccctggagttccatgataccacacgaacacagctttttgccttcgagctatcggggtaaagacctacaggaaaactactgtcgaaatcctcgaggggaagaagggggaccctggtgtttcacaagcaatccagaggtacgctacgaagtctgtgacattcctcagtgttcagaagttgaatgcatgacctgcaatggggagagttatcgaggtctcatggatcatacagaatcaggcaagatttgtcagcgctgggatcatcagacaccacaccggcacaaattcttgcctgaaagatatcccgacaagggctttgatgataattattgccgcaatcccgatggccagccgaggccatggtgctatactcttgaccctcacacccgctgggagtactgtgcaattaaaacatgcgctgacaatactatgaatgacactgatgttcctttggaaacaactgaatgcatccaaggtcaaggagaaggctacaggggcactgtcaataccatttggaatggaattccatgtcagcgttgggattctcagtatcctcacgagcatgacatgactcctgaaaatttcaagtgcaaggacctacgagaaaattactgccgaaatccagatgggtctgaatcaccctggtgttttaccactgatccaaacatccgagttggctactgctcccaaattccaaactgtgatatgtcacatggacaagattgttatcgtgggaatggcaaaaattatatgggcaacttatcccaaacaagatctggactaacatgttcaatgtgggacaagaacatggaagacttacatcgtcatatcttctgggaaccagatgcaagtaagctgaatgagaattactgccgaaatccagatgatgatgctcatggaccctggtgctacacgggaaatccactcattccttgggattattgccctatttctcgttgtgaaggtgataccacacctacaatagtcaatttagaccatcccgtaatatcttgtgccaaaacgaaacaattgcgagttgtaaatgggattccaacacgaacaaacataggatggatggttagtttgagatacagaaataaacatatctgcggaggatcattgataaaggagagttgggttcttactgcacgacagtgtttcccttctcgagacttgaaagattatgaagcttggcttggaattcatgatgtccacggaagaggagatgagaaatgcaaacaggttctcaatgtttcccagctggtatatggccctgaaggatcagatctggttttaatgaagcttgccaggcctgctgtcctggatgattttgttagtacgattgatttacctaattatggatgcacaattcctgaaaagaccagttgcagtgtttatggctggggctacactggattgatcaactatgatggcctattacgagtggcacatctctatataatgggaaatgagaaatgcagccagcatcatcgagggaaggtgactctgaatgagtctgaaatatgtgctggggctgaaaagattggatcaggaccatgtgagggggattatggtggcccacttgtttgtgagcaacataaaatgagaatggttcttggtgtcattgttcctggtcgtggatgtgccattccaaatcgtcctggtatttttgtccgagtagcatattatgcaaaatggatacacaaaattattttaacatataaggtaccacagtcataggaattctgcagatatccatcacactggcggccgctcgagcatgcatctagagggccctattctatagtgtcacctaaatgctagagctcgctgatcagcctcgactgtgccttctagttgccagccatctgttgtttgcccctcccccgtgccttccttgaccctggaaggtgccactcccactgtcctttcctaataaaatgaggaaattgcatcgcattgtctgagtaggtgtcattctattctggggggtggggtggggcaggacagcaagggggaggattgggaagacaatagcaggcatgctggggatgcggtgggctctatgg